European Patent Application EP 4 296 259 A1, published December 27, 2023. Title: New ceramide, method for preparing the new ceramide and its use. Applicant: LCS Biotech Co., Ltd. The sequence listing filed with the application follows.

SEQUENCE LISTING (8 sequences)

SEQ ID NO: 1 - DNA, 20 bp, Artificial Sequence
  GAPDH (F)
gagtcaacggatttggtcgt

SEQ ID NO: 2 - DNA, 20 bp, Artificial Sequence
  GAPDH (R)
ttgattttggagggatctcg

SEQ ID NO: 3 - DNA, 20 bp, Artificial Sequence
  SPTLC-1 (F)
gcgcgctacttggagaaaga

SEQ ID NO: 4 - DNA, 20 bp, Artificial Sequence
  SPTLC-1 (R)
tgttccaccgtgaccacaac

SEQ ID NO: 5 - DNA, 19 bp, Artificial Sequence
  SPTLC-2 (F)
agccgccaaagtccttgag

SEQ ID NO: 6 - DNA, 22 bp, Artificial Sequence
  SPTLC-2 (R)
cttgtccaggtttccaatttcc

SEQ ID NO: 7 - DNA, 22 bp, Artificial Sequence
  CER3 (F)
acattccacaaggcaaccattg

SEQ ID NO: 8 - DNA, 20 bp, Artificial Sequence
  CER3 (R)
ctcttgattccgccgactcc